European Patent Specification EP 3 344 264 B1, published March 15, 2023. Title: THREE-DIMENSIONAL DIFFERENTIATION OF EPIBLAST SPHEROIDS TO KIDNEY ORGANOIDS MODELS STAGE-SPECIFIC EPITHELIAL PHYSIOLOGY, MORPHOGENESIS, AND DISEASE. Applicant: THE BRIGHAM AND WOMEN'S HOSPITAL, INC. FREEDMAN, Benjamin S. BONVENTRE, Joseph V. The sequence listing filed with the application follows.

SEQUENCE LISTING (12 sequences)

SEQ ID NO: 1 - DNA, 23 bp, Artificial Sequence
  PODXL
gctacaccttcacaagcccgggg

SEQ ID NO: 2 - DNA, 23 bp, Artificial Sequence
  Exon 1 PKD2 Exon1
gcgtggagccgcgataaccccgg

SEQ ID NO: 3 - DNA, 23 bp, Artificial Sequence
  PKD1 Exon 36
gtgggtgcgagcttccccccggg

SEQ ID NO: 4 - DNA, 43 bp, Artificial Sequence
  PODXL WT
tccctggctacaccttcacaagcccggggatgaccaccaccct

SEQ ID NO: 5 - DNA, 43 bp, Artificial Sequence
  PODXL A1
tccctggctacaccttcacaagccccggggatgaccaccaccc

SEQ ID NO: 6 - DNA, 39 bp, Artificial Sequence
  PODXL A1
tccctggctacaccttcacaagccggatgaccaccaccc

SEQ ID NO: 7 - DNA, 21 bp, Artificial Sequence
  PKD1 WT
tgtgccccgcgtacggccacc

SEQ ID NO: 8 - DNA, 21 bp, Artificial Sequence
  PKD1 Al
tgtgccccggtacggccaccc

SEQ ID NO: 9 - DNA, 21 bp, Artificial Sequence
  PKD1 A2
tgtgccccgccgtacggccac

SEQ ID NO: 10 - DNA, 21 bp, Artificial Sequence
  PKD2 WT
gccgcgataaccccggcttcg

SEQ ID NO: 11 - DNA, 21 bp, Artificial Sequence
  PKD2 Al
gccgcgataaccccggcttca

SEQ ID NO: 12 - DNA, 21 bp, Artificial Sequence
  PKD2 A2
gccgcgataccccggcttcga